European Patent Application EP 4 582 560 A1, published July 9, 2025. Title: Differentially Methylated Region of ADHFE1 Gene, Kit, and Use thereof. Applicant: BGI GENOMICS CO., LTD. Application WO PCT/CN2022/116741, filed September 2, 2022. The sequence listing filed with the application follows.

SEQUENCE LISTING (105 sequences)

SEQ ID NO: 1 - DNA, 1366 bp, Homo sapiens
  source 1..1366: mol_type = genomic DNA
agtctaatcatggcaagttttaactattgatgtaagagttttaactattgattttgctttcatcaaaagcaaagccattcacacagtatttaacaaaaaccctcgggctctgctaggttcttgtttactgttaaaacagtttaaaggcagggtcttgatcacttaaaatactcttagaagggaaagtaacattttaaaggattaacagtggaaaaagaatatccctgttcctcttccttcccccaagtcctcaacatgtgaaaaatagagttgataagtaaggagatttaaggcagaacccgaggcctacggagcagttaccttctacggcaatttcaagggtggatggtgcgagcgccgctggggcagctggcgttctggttcttactccgtgggaaaatggccctgagcccgactggcttgaggcttagacaggtgaccccgcgaagcgggtgggcaggcgcggccgaggggcgggaggcgggcagcctccgtgattggccggcggagggggcggtgtagcgacccgaggagggaagaggactccaagcgccatggccgctgccgcccgagcccgggtcgcgtacttgctgaggcaactgcaacgcgcagcgtgagtgcggggccggcgggcgggcaggggaccgcagggtgcccacgcagccccctgggtgtgacccgctcagatcctgcgcagtcttctccgcttactttcaagaattcggagaatttggataccgccctgggctcccaccgcgcgccaggcggaacagcgaggtcacagagtgcgcgatgcagcctctcagggcgcagtgaggcagcctttactctgcttgtctaccgttaaagaaactgaggcccagagaggacctggtcccacatcgtagcaggcagtggagagcttggcacggtggccaagacaaattcatgtatgcaattgacacatatttattgggcatatattatgtgccaaaaactattctaggttctggggatacaaagatgaaaggctctggagcagtttgaggtctagtggggaatgggatgaggggacgaggctaaaaccggctatagcagactgggtgtagaagggaaggatggatgtgagaagtcgcagagtcacacttcctggcatgtacagggagtcagggtattcaatgtcatgacacgcctgcctcccagcagaaatgtgaggtacatcctggtcacctgataaatacttgctgactgtgcaagtgcacaagtctgcctgggaaacatggaaaagtttgagctcacaggtgcagatcagtaggaggaaaggcgagggactggcgaggaacgtcaggcagagagaagagcaacaccagcgatggagatgcagtcc

SEQ ID NO: 2 - DNA, 17 bp, synthetic construct
  source 1..17: mol_type = other DNA
tcgttggggtagttggc

SEQ ID NO: 3 - DNA, 24 bp, synthetic construct
  source 1..24: mol_type = other DNA
cctatctaaacctcaaaccaatcg

SEQ ID NO: 4 - DNA, 20 bp, synthetic construct
  source 1..20: mol_type = other DNA
gttttgggtttttatcgcgc

SEQ ID NO: 5 - DNA, 21 bp, synthetic construct
  source 1..21: mol_type = other DNA
gccctaaaaaactacatcgcg

SEQ ID NO: 6 - DNA, 22 bp, synthetic construct
  source 1..22: mol_type = other DNA
aggtttagataggtgatttcgc

SEQ ID NO: 7 - DNA, 16 bp, synthetic construct
  source 1..16: mol_type = other DNA
aaactacccgcctccc

SEQ ID NO: 8 - DNA, 22 bp, synthetic construct
  source 1..22: mol_type = other DNA
ttggcgttttggtttttatttc

SEQ ID NO: 9 - DNA, 26 bp, synthetic construct
  source 1..26: mol_type = other DNA
gatttaaggtagaattcgaggtttac

SEQ ID NO: 10 - DNA, 21 bp, synthetic construct
  source 1..21: mol_type = other DNA
cacgaaataaaaaccaaaacg

SEQ ID NO: 11 - DNA, 22 bp, synthetic construct
  source 1..22: mol_type = other DNA
cgtagttttttgggtgtgattc

SEQ ID NO: 12 - DNA, 22 bp, synthetic construct
  source 1..22: mol_type = other DNA
aaaacgatatccaaattctccg

SEQ ID NO: 13 - DNA, 24 bp, synthetic construct
  source 1..24: mol_type = other DNA
cgtattttgtgatttcgttgtttc

SEQ ID NO: 14 - DNA, 25 bp, synthetic construct
  source 1..25: mol_type = other DNA
aaaaattcgaaaaatttaaataccg

SEQ ID NO: 15 - DNA, 20 bp, synthetic construct
  source 1..20: mol_type = other DNA
cgtttgtttattcgtttcgc

SEQ ID NO: 16 - DNA, 20 bp, synthetic construct
  source 1..20: mol_type = other DNA
cgccgctaaaacaactaacg

SEQ ID NO: 17 - DNA, 21 bp, synthetic construct
  source 1..21: mol_type = other DNA
cgttttgagaggttgtatcgc

SEQ ID NO: 18 - DNA, 25 bp, synthetic construct
  source 1..25: mol_type = other DNA
gtttagggcggtatttaaatttttc

SEQ ID NO: 19 - DNA, 23 bp, synthetic construct
  source 1..23: mol_type = other DNA
atataacccgctcaaatcctacg

SEQ ID NO: 20 - DNA, 23 bp, synthetic construct
  source 1..23: mol_type = other DNA
tgtatcgcgtattttgtgatttc

SEQ ID NO: 21 - DNA, 21 bp, synthetic construct
  source 1..21: mol_type = other DNA
ccgcttactttcaaaaattcg

SEQ ID NO: 22 - DNA, 23 bp, synthetic construct
  source 1..23: mol_type = other DNA
ggtaattttaagggtggatggtg

SEQ ID NO: 23 - DNA, 23 bp, synthetic construct
  source 1..23: mol_type = other DNA
tcacctatctaaacctcaaacca

SEQ ID NO: 24 - DNA, 29 bp, synthetic construct
  source 1..29: mol_type = other DNA
ggggttatttgtttaagttttaagttagt

SEQ ID NO: 25 - DNA, 27 bp, synthetic construct
  source 1..27: mol_type = other DNA
aaacaattaccttctacracaatttca

SEQ ID NO: 26 - DNA, 25 bp, synthetic construct
  source 1..25: mol_type = other DNA
aagtaaggagatttaaggtagaatt

SEQ ID NO: 27 - DNA, 21 bp, synthetic construct
  source 1..21: mol_type = other DNA
ttaaaatcctcttccctcctc

SEQ ID NO: 28 - DNA, 30 bp, synthetic construct
  source 1..30: mol_type = other DNA
atatgtgaaaaatagagttgataagtaagg

SEQ ID NO: 29 - DNA, 22 bp, synthetic construct
  source 1..22: mol_type = other DNA
cttaaaatcctcttccctcctc

SEQ ID NO: 30 - DNA, 15 bp, synthetic construct
  source 1..15: mol_type = other DNA
gatggtgcgagcgtc

SEQ ID NO: 31 - DNA, 23 bp, synthetic construct
  source 1..23: mol_type = other DNA
ctatctaaacctcaaaccaatcg

SEQ ID NO: 32 - DNA, 15 bp, synthetic construct
  source 1..15: mol_type = other DNA
tacaccgccccctcc

SEQ ID NO: 33 - DNA, 16 bp, synthetic construct
  source 1..16: mol_type = other DNA
tccgccgaccaatcac

SEQ ID NO: 34 - DNA, 18 bp, synthetic construct
  source 1..18: mol_type = other DNA
ccgaactcgaacgacaac

SEQ ID NO: 35 - DNA, 32 bp, synthetic construct
  source 1..32: mol_type = other DNA
ayggtaattttaagggtggatggtgygagygt

SEQ ID NO: 36 - DNA, 30 bp, synthetic construct
  source 1..30: mol_type = other DNA
crccccctccrccraccaatcacraaaact

SEQ ID NO: 37 - DNA, 43 bp, synthetic construct
  source 1..43: mol_type = other DNA
aagtaaggagatttaaggtagaattygaggtttayggagtagt

SEQ ID NO: 38 - DNA, 39 bp, synthetic construct
  source 1..39: mol_type = other DNA
accataacrcttaaaatcctcttccctcctcraatcrct

SEQ ID NO: 39 - DNA, 29 bp, synthetic construct
  source 1..29: mol_type = other DNA
ggagatttaaggtagaattcgaggtttac

SEQ ID NO: 40 - DNA, 22 bp, synthetic construct
  source 1..22: mol_type = other DNA
ctcgaacgacaacgaccataac

SEQ ID NO: 41 - DNA, 23 bp, synthetic construct
  source 1..23: mol_type = other DNA
gaattcgaggtttacggagtagt

SEQ ID NO: 42 - DNA, 19 bp, synthetic construct
  source 1..19: mol_type = other DNA
ctcctcgaatcgctacacc

SEQ ID NO: 43 - DNA, 22 bp, synthetic construct
  source 1..22: mol_type = other DNA
tttaagggtggatggtgcgagc

SEQ ID NO: 44 - DNA, 19 bp, synthetic construct
  source 1..19: mol_type = other DNA
ctcaacaaatacgcgaccc

SEQ ID NO: 45 - DNA, 22 bp, synthetic construct
  source 1..22: mol_type = other DNA
cggttaattacggaggttgttc

SEQ ID NO: 46 - DNA, 25 bp, synthetic construct
  source 1..25: mol_type = other DNA
cctacgaaacaattaccttctacga

SEQ ID NO: 47 - DNA, 21 bp, synthetic construct
  source 1..21: mol_type = other DNA
aaaacaaaacccgaaacctac

SEQ ID NO: 48 - DNA, 23 bp, synthetic construct
  source 1..23: mol_type = other DNA
tagtaagtacgcgattcgggttc

SEQ ID NO: 49 - DNA, 27 bp, synthetic construct
  source 1..27: mol_type = other DNA
gaaacctacgaaacaattaccttctac

SEQ ID NO: 50 - DNA, 21 bp, synthetic construct
  source 1..21: mol_type = other DNA
cggagtagttattttttacgg

SEQ ID NO: 51 - DNA, 18 bp, synthetic construct
  source 1..18: mol_type = other DNA
aacgacaacgaccataac

SEQ ID NO: 52 - DNA, 24 bp, synthetic construct
  source 1..24: mol_type = other DNA
gttacaattacctcaacaaatacg

SEQ ID NO: 53 - DNA, 20 bp, synthetic construct
  source 1..20: mol_type = other DNA
ggtagaattcgaggtttacg

SEQ ID NO: 54 - DNA, 18 bp, synthetic construct
  source 1..18: mol_type = other DNA
tcttccctcctcgaatcg

SEQ ID NO: 55 - DNA, 19 bp, synthetic construct
  source 1..19: mol_type = other DNA
caatcacgaaaactacccg

SEQ ID NO: 56 - DNA, 17 bp, synthetic construct
  source 1..17: mol_type = other DNA
gaactcgaacgacaacg

SEQ ID NO: 57 - DNA, 18 bp, synthetic construct
  source 1..18: mol_type = other DNA
aactcgaacgacaacgac

SEQ ID NO: 58 - DNA, 25 bp, synthetic construct
  source 1..25: mol_type = other DNA
cgttacaattacctcaacaaatacg

SEQ ID NO: 59 - DNA, 22 bp, synthetic construct
  source 1..22: mol_type = other DNA
ttaaaatcctcttccctcctcg

SEQ ID NO: 60 - DNA, 17 bp, synthetic construct
  source 1..17: mol_type = other DNA
atcctcttccctcctcg

SEQ ID NO: 61 - DNA, 21 bp, synthetic construct
  source 1..21: mol_type = other DNA
aggtagaattcgaggtttacg

SEQ ID NO: 62 - DNA, 15 bp, synthetic construct
  source 1..15: mol_type = other DNA
tacccacccgcttcg

SEQ ID NO: 63 - DNA, 22 bp, synthetic construct
  source 1..22: mol_type = other DNA
tgggaaaatggttttgagttcg

SEQ ID NO: 64 - DNA, 21 bp, synthetic construct
  source 1..21: mol_type = other DNA
gagggaagaggattttaagcg

SEQ ID NO: 65 - DNA, 24 bp, synthetic construct
  source 1..24: mol_type = other DNA
ccaaaacgatatccaaattctccg

SEQ ID NO: 66 - DNA, 19 bp, synthetic construct
  source 1..19: mol_type = other DNA
ggatcgtagggtgtttacg

SEQ ID NO: 67 - DNA, 23 bp, synthetic construct
  source 1..23: mol_type = other DNA
ctacgccctaaaaaactacatcg

SEQ ID NO: 68 - DNA, 23 bp, synthetic construct
  source 1..23: mol_type = other DNA
gaattcggagaatttggatatcg

SEQ ID NO: 69 - DNA, 21 bp, synthetic construct
  source 1..21: mol_type = other DNA
aactctccactacctactacg

SEQ ID NO: 70 - DNA, 26 bp, synthetic construct
  source 1..26: mol_type = other DNA
gcgtatttgttgaggtaattgtaacg

SEQ ID NO: 71 - DNA, 22 bp, synthetic construct
  source 1..22: mol_type = other DNA
actctataacctcgctattccg

SEQ ID NO: 72 - DNA, 23 bp, synthetic construct
  source 1..23: mol_type = other DNA
aggagggaagaggattttaagcg

SEQ ID NO: 73 - DNA, 25 bp, synthetic construct
  source 1..25: mol_type = other DNA
cccaaaacgatatccaaattctccg

SEQ ID NO: 74 - DNA, 21 bp, synthetic construct
  source 1..21: mol_type = other DNA
ggggatcgtagggtgtttacg

SEQ ID NO: 75 - DNA, 27 bp, synthetic construct
  source 1..27: mol_type = other DNA
ctcactacgccctaaaaaactacatcg

SEQ ID NO: 76 - DNA, 24 bp, synthetic construct
  source 1..24: mol_type = other DNA
tcggttaattacggaggttgttcg

SEQ ID NO: 77 - DNA, 26 bp, synthetic construct
  source 1..26: mol_type = other DNA
aacctacgaaacaattaccttctacg

SEQ ID NO: 78 - DNA, 28 bp, synthetic construct
  source 1..28: mol_type = other DNA
gagtttagggcggtatttaaatttttcg

SEQ ID NO: 79 - DNA, 21 bp, synthetic construct
  source 1..21: mol_type = other DNA
aaactccaaacgccataaccg

SEQ ID NO: 80 - DNA, 22 bp, synthetic construct
  source 1..22: mol_type = other DNA
ttaagcgttatggtcgttgtcg

SEQ ID NO: 81 - DNA, 21 bp, synthetic construct
  source 1..21: mol_type = other DNA
gcgcgataaaaacccaaaacg

SEQ ID NO: 82 - DNA, 26 bp, synthetic construct
  source 1..26: mol_type = other DNA
tcaaaaccattttcccacgaaataaa

SEQ ID NO: 83 - DNA, 24 bp, synthetic construct
  source 1..24: mol_type = other DNA
ctctataacctcgctattccgcct

SEQ ID NO: 84 - DNA, 28 bp, synthetic construct
  source 1..28: mol_type = other DNA
cccacgaaataaaaaccaaaacgccaac

SEQ ID NO: 85 - DNA, 23 bp, synthetic construct
  source 1..23: mol_type = other DNA
actcaaaaccattttcccacgaa

SEQ ID NO: 86 - DNA, 25 bp, synthetic construct
  source 1..25: mol_type = other DNA
actcaaaaccattttcccacgaaat

SEQ ID NO: 87 - DNA, 27 bp, synthetic construct
  source 1..27: mol_type = other DNA
aacgaaaaacgccactacccgatacga

SEQ ID NO: 88 - DNA, 28 bp, synthetic construct
  source 1..28: mol_type = other DNA
aacgccactacccgatacgaactacacc

SEQ ID NO: 89 - DNA, 25 bp, synthetic construct
  source 1..25: mol_type = other DNA
aaaaaccaaaacgccaactacccca

SEQ ID NO: 90 - DNA, 24 bp, synthetic construct
  source 1..24: mol_type = other DNA
caaaacgccaactaccccaacgac

SEQ ID NO: 91 - DNA, 19 bp, synthetic construct
  source 1..19: mol_type = other DNA
tgcgagcgtcgttggggta

SEQ ID NO: 92 - DNA, 23 bp, synthetic construct
  source 1..23: mol_type = other DNA
tggtcgttgtcgttcgagttcgg

SEQ ID NO: 93 - DNA, 22 bp, synthetic construct
  source 1..22: mol_type = other DNA
cctcgctattccgcctaacgcg

SEQ ID NO: 94 - DNA, 24 bp, synthetic construct
  source 1..24: mol_type = other DNA
actacgcaaaatctaaacgaatca

SEQ ID NO: 95 - DNA, 22 bp, synthetic construct
  source 1..22: mol_type = other DNA
tatggtcgttgtcgttcgagtt

SEQ ID NO: 96 - DNA, 22 bp, synthetic construct
  source 1..22: mol_type = other DNA
tacgtaaacaccctacgatccc

SEQ ID NO: 97 - DNA, 20 bp, synthetic construct
  source 1..20: mol_type = other DNA
ttcgtttagattttgcgtag

SEQ ID NO: 98 - DNA, 23 bp, synthetic construct
  source 1..23: mol_type = other DNA
aacgatatccaaattctccgaat

SEQ ID NO: 99 - DNA, 23 bp, synthetic construct
  source 1..23: mol_type = other DNA
ttcgtttttcggtcgcgtttgtt

SEQ ID NO: 100 - DNA, 31 bp, synthetic construct
  source 1..31: mol_type = other DNA
atacgaacgccgctaaaacaactaacgttct

SEQ ID NO: 101 - DNA, 24 bp, synthetic construct
  source 1..24: mol_type = other DNA
taccgcccgaacccgaatcgcgta

SEQ ID NO: 102 - DNA, 19 bp, synthetic construct
  source 1..19: mol_type = other DNA
aagcggagaagattgcgta

SEQ ID NO: 103 - DNA, 23 bp, synthetic construct
  source 1..23: mol_type = other DNA
tttaggagtgagtggaagataga

SEQ ID NO: 104 - DNA, 23 bp, synthetic construct
  source 1..23: mol_type = other DNA
aaaccacaccatcctaattacct

SEQ ID NO: 105 - DNA, 23 bp, synthetic construct
  source 1..23: mol_type = other DNA
cccaaaacacatttcttccattc